European Patent Specification EP 2 972 353 B1, published February 22, 2023. Title: Improved Methods for Conducting Multiplexed Assays. Applicant: Meso Scale Technologies, LLC. The sequence listing filed with the application follows.

SEQUENCE LISTING (50 sequences)

SEQ ID NO: 1 - DNA, 12 bp, Artificial Sequence
  oligonucleotide
acatcggtagtt

SEQ ID NO: 2 - DNA, 12 bp, Artificial Sequence
  oligonucleotide
aactaccgatgt

SEQ ID NO: 3 - DNA, 12 bp, Artificial Sequence
  oligonucleotide
acgtcccagttg

SEQ ID NO: 4 - DNA, 12 bp, Artificial Sequence
  oligonucleotide
caactgggacgt

SEQ ID NO: 5 - DNA, 12 bp, Artificial Sequence
  oligonucleotide
agaagaagatcc

SEQ ID NO: 6 - DNA, 12 bp, Artificial Sequence
  oligonucleotide
ggatcttcttct

SEQ ID NO: 7 - DNA, 12 bp, Artificial Sequence
  oligonucleotide
aggttcagtgca

SEQ ID NO: 8 - DNA, 12 bp, Artificial Sequence
  oligonucleotide
tgcactgaacct

SEQ ID NO: 9 - DNA, 12 bp, Artificial Sequence
  oligonucleotide
atcaggatacgc

SEQ ID NO: 10 - DNA, 12 bp, Artificial Sequence
  oligonucleotide
gcgtatcctgat

SEQ ID NO: 11 - DNA, 12 bp, Artificial Sequence
  oligonucleotide
atcattaccacc

SEQ ID NO: 12 - DNA, 12 bp, Artificial Sequence
  oligonucleotide
ggtggtaatgat

SEQ ID NO: 13 - DNA, 12 bp, Artificial Sequence
  oligonucleotide
attaacgggagc

SEQ ID NO: 14 - DNA, 12 bp, Artificial Sequence
  oligonucleotide
gctcccgttaat

SEQ ID NO: 15 - DNA, 12 bp, Artificial Sequence
  oligonucleotide
cagaggtcttaa

SEQ ID NO: 16 - DNA, 12 bp, Artificial Sequence
  oligonucleotide
ttaagacctctg

SEQ ID NO: 17 - DNA, 12 bp, Artificial Sequence
  oligonucleotide
caggtgtccatt

SEQ ID NO: 18 - DNA, 12 bp, Artificial Sequence
  oligonucleotide
aatggacacctg

SEQ ID NO: 19 - DNA, 12 bp, Artificial Sequence
  oligonucleotide
catccaatccag

SEQ ID NO: 20 - DNA, 12 bp, Artificial Sequence
  oligonucleotide
ctggattggatg

SEQ ID NO: 21 - DNA, 12 bp, Artificial Sequence
  oligonucleotide
cctacgatatac

SEQ ID NO: 22 - DNA, 12 bp, Artificial Sequence
  oligonucleotide
gtatatcgtagg

SEQ ID NO: 23 - DNA, 12 bp, Artificial Sequence
  oligonucleotide
cgaatgtagagt

SEQ ID NO: 24 - DNA, 12 bp, Artificial Sequence
  oligonucleotide
actctacattcg

SEQ ID NO: 25 - DNA, 12 bp, Artificial Sequence
  oligonucleotide
cggtttgagata

SEQ ID NO: 26 - DNA, 12 bp, Artificial Sequence
  oligonucleotide
tatctcaaaccg

SEQ ID NO: 27 - DNA, 12 bp, Artificial Sequence
  oligonucleotide
cttacaacgcca

SEQ ID NO: 28 - DNA, 12 bp, Artificial Sequence
  oligonucleotide
tggcgttgtaag

SEQ ID NO: 29 - DNA, 12 bp, Artificial Sequence
  oligonucleotide
ctttctcggcac

SEQ ID NO: 30 - DNA, 12 bp, Artificial Sequence
  oligonucleotide
gtgccgagaaag

SEQ ID NO: 31 - DNA, 12 bp, Artificial Sequence
  oligonucleotide
gacataaagcga

SEQ ID NO: 32 - DNA, 12 bp, Artificial Sequence
  oligonucleotide
tcgctttatgtc

SEQ ID NO: 33 - DNA, 12 bp, Artificial Sequence
  oligonucleotide
gccatagtctct

SEQ ID NO: 34 - DNA, 12 bp, Artificial Sequence
  oligonucleotide
agagactatggc

SEQ ID NO: 35 - DNA, 12 bp, Artificial Sequence
  oligonucleotide
gctaattcacca

SEQ ID NO: 36 - DNA, 12 bp, Artificial Sequence
  oligonucleotide
tggtgaattagc

SEQ ID NO: 37 - DNA, 12 bp, Artificial Sequence
  oligonucleotide
ggtcgtgtttca

SEQ ID NO: 38 - DNA, 12 bp, Artificial Sequence
  oligonucleotide
tgaaacacgacc

SEQ ID NO: 39 - DNA, 12 bp, Artificial Sequence
  oligonucleotide
gttgattctgtc

SEQ ID NO: 40 - DNA, 12 bp, Artificial Sequence
  oligonucleotide
gacagaatcaac

SEQ ID NO: 41 - DNA, 12 bp, Artificial Sequence
  oligonucleotide
tacccggaataa

SEQ ID NO: 42 - DNA, 12 bp, Artificial Sequence
  oligonucleotide
ttattccgggta

SEQ ID NO: 43 - DNA, 12 bp, Artificial Sequence
  oligonucleotide
tgcttgacttgg

SEQ ID NO: 44 - DNA, 12 bp, Artificial Sequence
  oligonucleotide
ccaagtcaagca

SEQ ID NO: 45 - DNA, 12 bp, Artificial Sequence
  oligonucleotide
ttccacttaggg

SEQ ID NO: 46 - DNA, 12 bp, Artificial Sequence
  oligonucleotide
ccctaagtggaa

SEQ ID NO: 47 - DNA, 12 bp, Artificial Sequence
  oligonucleotide
ttgtctagcggc

SEQ ID NO: 48 - DNA, 12 bp, Artificial Sequence
  oligonucleotide
gccgctagacaa

SEQ ID NO: 49 - DNA, 12 bp, Artificial Sequence
  oligonucleotide
tttcccttgcta

SEQ ID NO: 50 - DNA, 12 bp, Artificial Sequence
  oligonucleotide
tagcaagggaaa